European Patent Specification EP 3 330 706 B1, published March 15, 2023. Title: Affinity Support and Method for Isolating Immunoglobrins. Applicant: JSR Corporation;JSR Life Sciences Corporation. The sequence listing filed with the application follows.

SEQUENCE LISTING (11 sequences)

SEQ ID NO: 1 - protein, 58 aa, Staphylococcus aureus [sequence omitted]

SEQ ID NO: 2 - protein, 58 aa, Staphylococcus aureus [sequence omitted]

SEQ ID NO: 3 - protein, 58 aa, Staphylococcus aureus
  Protein A, C domain
ADNKFNKEQQNAFYEILHLPNLTEEQRNGFIQSLKDDPSVSKEILAEAKKLNDAQAPK

SEQ ID NO: 4 - protein, 242 aa, Staphylococcus aureus
AQGTVDNKFNKEQQNAFYEILHLPNLTEEQRNAFIQSLKDDPSVSKEILAEAKKLNDAQAPKEFVDNKFNKEQQNAFYEILHLPNLTEEQRNAFIQSLKDDPSVSKEILAEAKKLNDAQAPKEFVDNKFNKEQQNAFYEILHLPNLTEEQRNAFIQSLKDDPSVSKEILAEAKKLNDAQAPKELVDNKFNKEQQNAFYEILHLPNLTEEQRNAFIQSLKDDPSVSKEILAEAKKLNDAQAPK

SEQ ID NO: 5 - protein, 243 aa, Staphylococcus aureus
AQGTVDNKFNKEQQNAFYEILHLPNLTEEQRNAFIQSLKDDPSVSKEILAEAKKLNDAQAPKEFVDNKFNKEQQNAFYEILHLPNLTEEQRNAFIQSLKDDPSVSKEILAEAKKLNDAQAPKEFVDNKFNKEQQNAFYEILHLPNLTEEQRNAFIQSLKDDPSVSKEILAEAKKLNDAQAPKELVDNKFNKEQQNAFYEILHLPNLTEEQRNAFIQSLKDDPSVSKEILAEAKKLNDAQAPKC

SEQ ID NO: 6 - protein, 241 aa, Staphylococcus aureus
VDNKFNKEQQNAFYEILHLPNLTEEQRNAFIQSLKDDPSVSKEILAEAKKLNDAQAPKEFVDNKFNKEQQNAFYEILHLPNLTEEQRNAFIQSLKDDPSVSKEILAEAKKLNDAQAPKEFVDNKFNKEQQNAFYEILHLPNLTEEQRNAFIQSLKDDPSVSKEILAEAKKLNDAQAPKELVDNKFNKEQQNAFYEILHLPNLTEEQRNAFIQSLKDDPSVSKEILAEAKKLNDAQAPKKKK

SEQ ID NO: 7 - protein, 249 aa, Staphylococcus aureus
AQGTVDNKFNKEQQNAFYEILHLPNLTEEQRNAFIQSLKDDPSVSKEILAEAKKLNDAQAPKEFVDNKFNKEQQNAFYEILHLPNLTEEQRNAFIQSLKDDPSVSKEILAEAKKLNDAQAPKEFVDNKFNKEQQNAFYEILHLPNLTEEQRNAFIQSLKDDPSVSKEILAEAKKLNDAQAPKELVDNKFNKEQQNAFYEILHLPNLTEEQRNAFIQSLKDDPSVSKEILAEAKKLNDAQAPKPPPPPPC

SEQ ID NO: 8 - protein, 252 aa, Staphylococcus aureus
AQGTVDNKFNKEQQNAFYEILHLPNLTEEQRNAFIQSLKDDPSVSKEILAEAKKLNDAQAPKEFVDNKFNKEQQNAFYEILHLPNLTEEQRNAFIQSLKDDPSVSKEILAEAKKLNDAQAPKEFVDNKFNKEQQNAFYEILHLPNLTEEQRNAFIQSLKDDPSVSKEILAEAKKLNDAQAPKELVDNKFNKEQQNAFYEILHLPNLTEEQRNAFIQSLKDDPSVSKEILAEAKKLNDAQAPKPPPPPPPPPC

SEQ ID NO: 9 - protein, 255 aa, Staphylococcus aureus
AQGTVDNKFNKEQQNAFYEILHLPNLTEEQRNAFIQSLKDDPSVSKEILAEAKKLNDAQAPKEFVDNKFNKEQQNAFYEILHLPNLTEEQRNAFIQSLKDDPSVSKEILAEAKKLNDAQAPKEFVDNKFNKEQQNAFYEILHLPNLTEEQRNAFIQSLKDDPSVSKEILAEAKKLNDAQAPKELVDNKFNKEQQNAFYEILHLPNLTEEQRNAFIQSLKDDPSVSKEILAEAKKLNDAQAPKPPPPPPPPPPPPC

SEQ ID NO: 10 - protein, 257 aa, Staphylococcus aureus
VDNKFNKEQQNAFYEILHLPNLTEEQRNAFIQSLKDDPSVSKEILAEAKKLNDAQAPKEFVDNKFNKEQQNAFYEILHLPNLTEEQRNAFIQSLKDDPSVSKEILAEAKKLNDAQAPKEFVDNKFNKEQQNAFYEILHLPNLTEEQRNAFIQSLKDDPSVSKEILAEAKKLNDAQAPKELVDNKFNKEQQNAFYEILHLPNLTEEQRNAFIQSLKDDPSVSKEILAEAKKLNDAQAPKPPPPPPPPPPPPPPPPPPC

SEQ ID NO: 11 - protein, 259 aa, Staphylococcus aureus
VDNKFNKEQQNAFYEILHLPNLTEEQRNAFIQSLKDDPSVSKEILAEAKKLNDAQAPKEFVDNKFNKEQQNAFYEILHLPNLTEEQRNAFIQSLKDDPSVSKEILAEAKKLNDAQAPKEFVDNKFNKEQQNAFYEILHLPNLTEEQRNAFIQSLKDDPSVSKEILAEAKKLNDAQAPKELVDNKFNKEQQNAFYEILHLPNLTEEQRNAFIQSLKDDPSVSKEILAEAKKLNDAQAPKPPPPPPPPPPPPPPPPPPKKK